European Patent Specification EP 3 670 654 B1, published October 1, 2025. Title: XYLANASE MUTANT. Applicant: QINGDAO VLAND BIOTECH GROUP CO.,LTD. The sequence listing filed with the application follows.

SEQUENCE LISTING (26 sequences)

SEQ ID NO: 1 - protein, 189 aa, Xyn
TIQPGTGYNNGYFYSYWNDGHGGVTYTNGPGGQFSVNWSNSGNFVGGKGWQPGTKNKVINFSGSYNPNGNSYLSVYGWSRNPLIEYYIVENFGTYNPSTGATKLGEVTSDGSVYDIYRTQRVNQPSIIGTATFYQYWSVRRNHRSSGSVNTANHFNAWAQQGLTLGTMDYQIVAVEGYFSSGSASITVS

SEQ ID NO: 2 - DNA, 567 bp, Xyn
actattcaacctggaactggatacaataacggttatttctactcttactggaacgatggacatggaggtgtcacatacactaacggtccaggtggacaattctcagttaattggtctaactcaggaaatttcgtcggaggtaaaggatggcaaccaggaactaagaataaggtcattaacttctcaggttcatataatccaaacggaaactcctacttgtccgtttacggttggtcccgtaaccctttgatcgaatattacattgttgaaaacttcggtacttataatccttccaccggagccactaagctgggtgaagtcacctctgatggttcagtttatgatatatatagaacacaacgtgttaatcaaccatccatcatcggtacagctacattttaccaatattggtctgttaggcgtaaccatcgtagctccggttccgtcaacaccgcaaatcatttcaatgcttgggcccaacaaggactgaccttaggtactatggattatcaaatcgtcgctgtcgaaggatacttctcctctggatctgcctctatcacagtctca

SEQ ID NO: 3 - protein, 189 aa, Artificial
TIQPGTGYNNGYFYSYWNDGHGGVTYTNGPGGCFSVNWSNSGNFVGGKGWQPGTKNKVINFSGSYNPNGNSYLSVYGWSRNPLIEYYIVENFGTYNPSTGATKLGEVTCDGSVYDIYRTQRVNQPSIIGTATFYQYWSVRRNHRSSGSVNTACHFNAWAQQGLTLGTMDYQIVAVEGYFSSGSASICVS

SEQ ID NO: 4 - DNA, 567 bp, Artificial
actattcaacctggaactggatacaataacggttatttctactcttactggaacgatggacatggaggtgtcacatacactaacggtccaggtggatgtttctcagttaattggtctaactcaggaaatttcgtcggaggtaaaggatggcaaccaggaactaagaataaggtcattaacttctcaggttcatataatccaaacggaaactcctacttgtccgtttacggttggtcccgtaaccctttgatcgaatattacattgttgaaaacttcggtacttataatccttccaccggagccactaagctgggtgaagtcacctgtgatggttcagtttatgatatatatagaacacaacgtgttaatcaaccatccatcatcggtacagctacattttaccaatattggtctgttaggcgtaaccatcgtagctccggttccgtcaacaccgcatgtcatttcaatgcttgggcccaacaaggactgaccttaggtactatggattatcaaatcgtcgctgtcgaaggatacttctcctctggatctgcctctatctgtgtctca

SEQ ID NO: 5 - protein, 189 aa, Artificial
CIQPGTGYNNGYFYSYWNDGHGGVTYCNGPGGCFSVNWSNSGNFVGGKGWQPGTKNKVINFSGSYNPNGNSYLSVYGWSRNPLIEYYIVENFGTYNPSTGATKLGEVTCDGSVYDIYRTQRVNQPSIIGTATFYQYWSVRRNHRSSGSVNTACHFNAWAQQGLTLGTMDYQIVAVEGYFSSGSASICVS

SEQ ID NO: 6 - DNA, 567 bp, Artificial
tgtattcaacctggaactggatacaataacggttatttctactcttactggaacgatggacatggaggtgtcacatactgtaacggtccaggtggatgtttctcagttaattggtctaactcaggaaatttcgtcggaggtaaaggatggcaaccaggaactaagaataaggtcattaacttctcaggttcatataatccaaacggaaactcctacttgtccgtttacggttggtcccgtaaccctttgatcgaatattacattgttgaaaacttcggtacttataatccttccaccggagccactaagctgggtgaagtcacctgtgatggttcagtttatgatatatatagaacacaacgtgttaatcaaccatccatcatcggtacagctacattttaccaatattggtctgttaggcgtaaccatcgtagctccggttccgtcaacaccgcatgtcatttcaatgcttgggcccaacaaggactgaccttaggtactatggattatcaaatcgtcgctgtcgaaggatacttctcctctggatctgcctctatctgtgtctca

SEQ ID NO: 7 - protein, 189 aa, Artificial
TIQPGTGYNNGYFYSYWNDGHGGVTYTNGPGGCFSVNWSNSGNFVGGKGWNPGTKNKVINFSGSYNPNGNSYLSVYGWSRNPLIEYYIVENFGTYNPSTGATKLGEVTCDGSVYDIYRTQRVNQPSIIGTATFYQYWSVRRNHRSSGSVNTACHFNAWAQQGLTLGTMDYQIVAVEGYFSSGSASICVS

SEQ ID NO: 8 - DNA, 567 bp, Artificial
actattcaacctggaactggatacaataacggttatttctactcttactggaacgatggacatggaggtgtcacatacactaacggtccaggtggatgtttctcagttaattggtctaactcaggaaatttcgtcggaggtaaaggatggaacccaggaactaagaataaggtcattaacttctcaggttcatataatccaaacggaaactcctacttgtccgtttacggttggtcccgtaaccctttgatcgaatattacattgttgaaaacttcggtacttataatccttccaccggagccactaagctgggtgaagtcacctgtgatggttcagtttatgatatatatagaacacaacgtgttaatcaaccatccatcatcggtacagctacattttaccaatattggtctgttaggcgtaaccatcgtagctccggttccgtcaacaccgcatgtcatttcaatgcttgggcccaacaaggactgaccttaggtactatggattatcaaatcgtcgctgtcgaaggatacttctcctctggatctgcctctatctgtgtctca

SEQ ID NO: 9 - protein, 189 aa, Artificial
TIQPGTGYNNGYFYSYWNDGHGGVTYTNGPGGCFSVNWSNSGNFVGGKGWQPGTKNKVINFSGSYNPNGNSYLSVYGWSRNPLIEYYIVENFGTYNPSTGATKLGEVTCDGSVYDIYRTQRVNQPSIIGTATFYQYWSVRRNKRSSGSVNTACHFNAWAQQGLTLGTMDYQIVAVEGYFSSGSASICVS

SEQ ID NO: 10 - DNA, 567 bp, Artificial
actattcaacctggaactggatacaataacggttatttctactcttactggaacgatggacatggaggtgtcacatacactaacggtccaggtggatgtttctcagttaattggtctaactcaggaaatttcgtcggaggtaaaggatggcaaccaggaactaagaataaggtcattaacttctcaggttcatataatccaaacggaaactcctacttgtccgtttacggttggtcccgtaaccctttgatcgaatattacattgttgaaaacttcggtacttataatccttccaccggagccactaagctgggtgaagtcacctgtgatggttcagtttatgatatatatagaacacaacgtgttaatcaaccatccatcatcggtacagctacattttaccaatattggtctgttaggcgtaacaagcgtagctccggttccgtcaacaccgcatgtcatttcaatgcttgggcccaacaaggactgaccttaggtactatggattatcaaatcgtcgctgtcgaaggatacttctcctctggatctgcctctatctgtgtctca

SEQ ID NO: 11 - protein, 189 aa, Artificial
TIQPGTGYNNGYFYSYWNDGHGGVTYTNGPGGCFSVNWSNSGNFVGGKGWQPGTKNKVINFSGSYNPNGNSYLSVYGWSRNPLIEYYIVENFGTYNPSTGATKLGEVTCDGSVYDIYRTQRVNQPSIIGTATFYQYWSVRRNHRSSGSVNTACHFNAWAQFGLTLGTMDYQIVAVEGYFSSGSASICVS

SEQ ID NO: 12 - DNA, 567 bp, Artificial
actattcaacctggaactggatacaataacggttatttctactcttactggaacgatggacatggaggtgtcacatacactaacggtccaggtggatgtttctcagttaattggtctaactcaggaaatttcgtcggaggtaaaggatggcaaccaggaactaagaataaggtcattaacttctcaggttcatataatccaaacggaaactcctacttgtccgtttacggttggtcccgtaaccctttgatcgaatattacattgttgaaaacttcggtacttataatccttccaccggagccactaagctgggtgaagtcacctgtgatggttcagtttatgatatatatagaacacaacgtgttaatcaaccatccatcatcggtacagctacattttaccaatattggtctgttaggcgtaaccatcgtagctccggttccgtcaacaccgcatgtcatttcaatgcttgggcccaattcggactgaccttaggtactatggattatcaaatcgtcgctgtcgaaggatacttctcctctggatctgcctctatctgtgtctca

SEQ ID NO: 13 - protein, 189 aa, Artificial
TIQPGTGYNNGYFYSYWNDGHGGVTYTNGPGGCFSVNWSNSGNFVGGKGWNPGTKNKVINFSGSYNPNGNSYLSVYGWSRNPLIEYYIVENFGTYNPSTGATKLGEVTCDGSVYDIYRTQRVNQPSIIGTATFYQYWSVRRNKRSSGSVNTACHFNAWAQQGLTLGTMDYQIVAVEGYFSSGSASICVS

SEQ ID NO: 14 - DNA, 567 bp, Artificial
actattcaacctggaactggatacaataacggttatttctactcttactggaacgatggacatggaggtgtcacatacactaacggtccaggtggatgtttctcagttaattggtctaactcaggaaatttcgtcggaggtaaaggatggaacccaggaactaagaataaggtcattaacttctcaggttcatataatccaaacggaaactcctacttgtccgtttacggttggtcccgtaaccctttgatcgaatattacattgttgaaaacttcggtacttataatccttccaccggagccactaagctgggtgaagtcacctgtgatggttcagtttatgatatatatagaacacaacgtgttaatcaaccatccatcatcggtacagctacattttaccaatattggtctgttaggcgtaacaagcgtagctccggttccgtcaacaccgcatgtcatttcaatgcttgggcccaacaaggactgaccttaggtactatggattatcaaatcgtcgctgtcgaaggatacttctcctctggatctgcctctatctgtgtctca

SEQ ID NO: 15 - protein, 189 aa, Artificial
TIQPGTGYNNGYFYSYWNDGHGGVTYTNGPGGCFSVNWSNSGNFVGGKGWQPGTKNKVINFSGSYNPNGNSYLSVYGWSRNPLIEYYIVENFGTYNPSTGATKLGEVTCDGSVYDIYRTQRVNQPSIIGTATFYQYWSVRRNKRSSGSVNTACHFNAWAQFGLTLGTMDYQIVAVEGYFSSGSASICVS

SEQ ID NO: 16 - DNA, 567 bp, Artificial
actattcaacctggaactggatacaataacggttatttctactcttactggaacgatggacatggaggtgtcacatacactaacggtccaggtggatgtttctcagttaattggtctaactcaggaaatttcgtcggaggtaaaggatggcaaccaggaactaagaataaggtcattaacttctcaggttcatataatccaaacggaaactcctacttgtccgtttacggttggtcccgtaaccctttgatcgaatattacattgttgaaaacttcggtacttataatccttccaccggagccactaagctgggtgaagtcacctgtgatggttcagtttatgatatatatagaacacaacgtgttaatcaaccatccatcatcggtacagctacattttaccaatattggtctgttaggcgtaacaagcgtagctccggttccgtcaacaccgcatgtcatttcaatgcttgggcccaattcggactgaccttaggtactatggattatcaaatcgtcgctgtcgaaggatacttctcctctggatctgcctctatctgtgtctca

SEQ ID NO: 17 - protein, 189 aa, Artificial
TIQPGTGYNNGYFYSYWNDGHGGVTYTNGPGGCFSVNWSNSGNFVGGKGWNPGTKNKVINFSGSYNPNGNSYLSVYGWSRNPLIEYYIVENFGTYNPSTGATKLGEVTCDGSVYDIYRTQRVNQPSIIGTATFYQYWSVRRNHRSSGSVNTACHFNAWAQFGLTLGTMDYQIVAVEGYFSSGSASICVS

SEQ ID NO: 18 - DNA, 567 bp, Artificial
actattcaacctggaactggatacaataacggttatttctactcttactggaacgatggacatggaggtgtcacatacactaacggtccaggtggatgtttctcagttaattggtctaactcaggaaatttcgtcggaggtaaaggatggaacccaggaactaagaataaggtcattaacttctcaggttcatataatccaaacggaaactcctacttgtccgtttacggttggtcccgtaaccctttgatcgaatattacattgttgaaaacttcggtacttataatccttccaccggagccactaagctgggtgaagtcacctgtgatggttcagtttatgatatatatagaacacaacgtgttaatcaaccatccatcatcggtacagctacattttaccaatattggtctgttaggcgtaaccatcgtagctccggttccgtcaacaccgcatgtcatttcaatgcttgggcccaattcggactgaccttaggtactatggattatcaaatcgtcgctgtcgaaggatacttctcctctggatctgcctctatctgtgtctca

SEQ ID NO: 19 - protein, 189 aa, Artificial
TIQPGTGYNNGYFYSYWNDGHGGVTYTNGPGGCFSVNWSNSGNFVGGKGWNPGTKNKVINFSGSYNPNGNSYLSVYGWSRNPLIEYYIVENFGTYNPSTGATKLGEVTCDGSVYDIYRTQRVNQPSIIGTATFYQYWSVRRNKRSSGSVNTACHFNAWAQFGLTLGTMDYQIVAVEGYFSSGSASICVS

SEQ ID NO: 20 - DNA, 567 bp, Artificial
actattcaacctggaactggatacaataacggttatttctactcttactggaacgatggacatggaggtgtcacatacactaacggtccaggtggatgtttctcagttaattggtctaactcaggaaatttcgtcggaggtaaaggatggaacccaggaactaagaataaggtcattaacttctcaggttcatataatccaaacggaaactcctacttgtccgtttacggttggtcccgtaaccctttgatcgaatattacattgttgaaaacttcggtacttataatccttccaccggagccactaagctgggtgaagtcacctgtgatggttcagtttatgatatatatagaacacaacgtgttaatcaaccatccatcatcggtacagctacattttaccaatattggtctgttaggcgtaacaagcgtagctccggttccgtcaacaccgcatgtcatttcaatgcttgggcccaattcggactgaccttaggtactatggattatcaaatcgtcgctgtcgaaggatacttctcctctggatctgcctctatctgtgtctca

SEQ ID NO: 21 - protein, 188 aa, Artificial
CIQPGTGYNNGYFYSYWNDGHGGVTYCNGPGGCFSVNWSNSGNFVGGKGWNPGTKNKVINFSGSYNPNGNSYLSVYGWSRNPLIEYYIVENFGTYNPSTGATKLGEVTCDGSVYDIYRTQRVNQPSIIGTATFYQYWSVRRNHRSSGSVNTACHFNAWAQQGLTLGTMDYQIVAVEGYFSSGSASICV

SEQ ID NO: 22 - DNA, 567 bp, Artificial
tgtattcaacctggaactggatacaataacggttatttctactcttactggaacgatggacatggaggtgtcacatactgtaacggtccaggtggatgtttctcagttaattggtctaactcaggaaatttcgtcggaggtaaaggatggaacccaggaactaagaataaggtcattaacttctcaggttcatataatccaaacggaaactcctacttgtccgtttacggttggtcccgtaaccctttgatcgaatattacattgttgaaaacttcggtacttataatccttccaccggagccactaagctgggtgaagtcacctgtgatggttcagtttatgatatatatagaacacaacgtgttaatcaaccatccatcatcggtacagctacattttaccaatattggtctgttaggcgtaaccatcgtagctccggttccgtcaacaccgcatgtcatttcaatgcttgggcccaacaaggactgaccttaggtactatggattatcaaatcgtcgctgtcgaaggatacttctcctctggatctgcctctatctgtgtctca

SEQ ID NO: 23 - protein, 189 aa, Artificial
CIQPGTGYNNGYFYSYWNDGHGGVTYCNGPGGCFSVNWSNSGNFVGGKGWQPGTKNKVINFSGSYNPNGNSYLSVYGWSRNPLIEYYIVENFGTYNPSTGATKLGEVTCDGSVYDIYRTQRVNQPSIIGTATFYQYWSVRRNKRSSGSVNTACHFNAWAQQGLTLGTMDYQIVAVEGYFSSGSASICVS

SEQ ID NO: 24 - DNA, 567 bp, Artificial
tgtattcaacctggaactggatacaataacggttatttctactcttactggaacgatggacatggaggtgtcacatactgtaacggtccaggtggatgtttctcagttaattggtctaactcaggaaatttcgtcggaggtaaaggatggcaaccaggaactaagaataaggtcattaacttctcaggttcatataatccaaacggaaactcctacttgtccgtttacggttggtcccgtaaccctttgatcgaatattacattgttgaaaacttcggtacttataatccttccaccggagccactaagctgggtgaagtcacctgtgatggttcagtttatgatatatatagaacacaacgtgttaatcaaccatccatcatcggtacagctacattttaccaatattggtctgttaggcgtaacaagcgtagctccggttccgtcaacaccgcatgtcatttcaatgcttgggcccaacaaggactgaccttaggtactatggattatcaaatcgtcgctgtcgaaggatacttctcctctggatctgcctctatctgtgtctca

SEQ ID NO: 25 - protein, 189 aa, Artificial
CIQPGTGYNNGYFYSYWNDGHGGVTYCNGPGGCFSVNWSNSGNFVGGKGWQPGTKNKVINFSGSYNPNGNSYLSVYGWSRNPLIEYYIVENFGTYNPSTGATKLGEVTCDGSVYDIYRTQRVNQPSIIGTATFYQYWSVRRNHRSSGSVNTACHFNAWAQFGLTLGTMDYQIVAVEGYFSSGSASICVS

SEQ ID NO: 26 - DNA, 567 bp, Artificial
tgtattcaacctggaactggatacaataacggttatttctactcttactggaacgatggacatggaggtgtcacatactgtaacggtccaggtggatgtttctcagttaattggtctaactcaggaaatttcgtcggaggtaaaggatggcaaccaggaactaagaataaggtcattaacttctcaggttcatataatccaaacggaaactcctacttgtccgtttacggttggtcccgtaaccctttgatcgaatattacattgttgaaaacttcggtacttataatccttccaccggagccactaagctgggtgaagtcacctgtgatggttcagtttatgatatatatagaacacaacgtgttaatcaaccatccatcatcggtacagctacattttaccaatattggtctgttaggcgtaaccatcgtagctccggttccgtcaacaccgcatgtcatttcaatgcttgggcccaaaacggactgaccttaggtactatggattatcaaatcgtcgctgtcgaaggatacttctcctctggatctgcctctatctgtgtctca